European Patent Application EP 4 269 429 A1, published November 1, 2023. Title: Novel peptides capable of inhibiting TGF-beta signaling and uses thereof. Applicant: Korea Institute of Science and Technology. The sequence listing filed with the application follows.

SEQUENCE LISTING (18 sequences)

SEQ ID NO: 1 - protein, 15 aa, Artificial Sequence
  P1
FCLGPCPYIWSLDTA

SEQ ID NO: 2 - protein, 14 aa, Artificial Sequence
  P2
FCLGPCPYIWCLDT

SEQ ID NO: 3 - protein, 14 aa, Artificial Sequence
  P3
FSLGPSPYIWSLDT

SEQ ID NO: 4 - protein, 15 aa, Artificial Sequence
  P4
FCLGPCPYIWSLDTF

SEQ ID NO: 5 - protein, 15 aa, Artificial Sequence
  P5
FCLGPCPYIWCLDTF

SEQ ID NO: 6 - protein, 18 aa, Artificial Sequence
  P6
FCLGPCPYIWSLDTVLSL

SEQ ID NO: 7 - protein, 18 aa, Artificial Sequence
  P7
FCLGPCPYIWCLDTVLSL

SEQ ID NO: 8 - protein, 18 aa, Artificial Sequence
  P8
FCLGPCPYIWCLDTVLSF

SEQ ID NO: 9 - protein, 10 aa, Artificial Sequence
  P9
AHCSCDSRDN

SEQ ID NO: 10 - protein, 10 aa, Artificial Sequence
  P10
AHCSCDGAFA

SEQ ID NO: 11 - protein, 14 aa, Artificial Sequence
  P11
TIVYYVGRKPKVEQ

SEQ ID NO: 12 - protein, 14 aa, Artificial Sequence
  P12
TIVYYVGLKPKVEQ

SEQ ID NO: 13 - protein, 14 aa, Artificial Sequence
  P13
TIVYYVHIKPKVEQ

SEQ ID NO: 14 - protein, 14 aa, Artificial Sequence
  P14
TIVYYVVIKPKVEQ

SEQ ID NO: 15 - protein, 14 aa, Artificial Sequence
  P144
TSLDASIWAMMQNA

SEQ ID NO: 16 - protein, 14 aa, Artificial Sequence
  peptide 1
  MISC_FEATURE (2): Xaa is cysteine or serine
  MISC_FEATURE (6): Xaa is cysteine or serine
  MISC_FEATURE (11): Xaa is cysteine or serine
FXLGPXPYIWXLDT

SEQ ID NO: 17 - protein, 6 aa, Artificial Sequence
  peptide 2
AHCSCD

SEQ ID NO: 18 - protein, 14 aa, Artificial Sequence
  peptide 3
  MISC_FEATURE (7): Xaa is glycine, histidine or valine
  MISC_FEATURE (8): Xaa is arginine, leucine or isoleucine
TIVYYVXXKPKVEQ